European Patent Application EP 4 394 047 A1, published July 3, 2024. Title: Méthode pour contrôler la qualité d'une amplification LAMP et kit utilisé à cet effet. Applicant: Commissariat a l'Energie Atomique et aux Energies Alternatives. Application EP EP23XXXXXX, filed December 21, 2023. The sequence listing filed with the application follows.

SEQUENCE LISTING (9 sequences)

SEQ ID NO: 1 - DNA, 162 bp, synthetic construct
  source 1..162: mol_type = other DNA
ggttggtgtggttggttttttttttcggatccaagacgcggtttatcgtgcagtacgccaacctttctcaataaaccgcgtcttggatccgtgacatctctgagttatatctttccccccctcactgaccctccttcgggggaaagatataactcagagatg

SEQ ID NO: 2 - DNA, 87 bp, synthetic construct
  source 1..87: mol_type = other DNA
cggcagtacgccaacctttctcaataaaccgcgtcttggatccgcatctctgagttatatctttccccccctcactgaccctccttc

SEQ ID NO: 3 - DNA, 113 bp, synthetic construct
  source 1..113: mol_type = other DNA
cgtgcagtacgccaacctttctcaataaaccgcgtcttggatccgcatctctgagttatatctttccccccctcactgaccctccttcgggggaaagatataactcagagatg

SEQ ID NO: 4 - DNA, 112 bp, synthetic construct
  source 1..112: mol_type = other DNA
cggatccaagacgcggtttatcgtgcagtacgccaacctttctcaataaaccgcgtcttggatccgtgacatctctgagttatatctttccccccctcactgaccctccttc

SEQ ID NO: 5 - DNA, 45 bp, synthetic construct
  source 1..45: mol_type = other DNA
cggatccaagacgcggtttatcgtgcagtacgccaacctttctca

SEQ ID NO: 6 - DNA, 43 bp, synthetic construct
  source 1..43: mol_type = other DNA
catctctgagttatatctttcccccgaaggagggtcagtgagg

SEQ ID NO: 7 - DNA, 147 bp, synthetic construct
  source 1..147: mol_type = other DNA
ggttggtgtggttggttttttttttagagcagcagaagtggcacaggtgattgtgaagaagaagagtgtgccacttctgctgctctttatcaacctgaagaagagcaggcagtgaggacaatcagttcttgctcttcttcaggttga

SEQ ID NO: 8 - DNA, 41 bp, synthetic construct
  source 1..41: mol_type = other DNA
agagcagcagaagtggcacaggtgattgtgaagaagaagag

SEQ ID NO: 9 - DNA, 40 bp, synthetic construct
  source 1..40: mol_type = other DNA
tcaacctgaagaagagcaagaactgattgtcctcactgcc